European Patent Application EP 4 122 485 A1, published January 25, 2023. Title: CONNEXIN 43 FOR USE IN THE TREATMENT OF RETINOBLASTOMA PROTEIN POSITIVE TUMOURS. Applicant: Fundación Profesor Novoa Santos Servizo Galego de Saúde. The sequence listing filed with the application follows.

SEQUENCE LISTING (14 sequences)

SEQ ID NO: 1 - DNA, 20 bp, Artificial sequence
  Artificial sequence
gactctcagggtcgaaaacg

SEQ ID NO: 2 - DNA, 21 bp, Artificial sequence
  Artificial sequence
gccagggtatgtacatgagga

SEQ ID NO: 3 - DNA, 20 bp, Artificial sequence
  Artificial sequence
acatgggtgactggagcgcc

SEQ ID NO: 4 - DNA, 20 bp, Artificial sequence
  Artificial sequence
atgatctgcaggacccagaa

SEQ ID NO: 5 - DNA, 21 bp, Artificial sequence
  Artificial sequence
cgaatctccgaccaccactac

SEQ ID NO: 6 - DNA, 20 bp, Artificial sequence
  Artificial sequence
tccatggccacaacaactga

SEQ ID NO: 7 - DNA, 17 bp, Artificial sequence
  Artificial sequence
tgtagccgccccacaca

SEQ ID NO: 8 - DNA, 22 bp, Artificial sequence
  Artificial sequence
ggatgtaccgaatttgtttgta

SEQ ID NO: 9 - DNA, 20 bp, Artificial sequence
  Artificial sequence
ttggcagccttcctgatttc

SEQ ID NO: 10 - DNA, 23 bp, Artificial sequence
  Artificial sequence
tctttagcactccttggcaaaac

SEQ ID NO: 11 - DNA, 20 bp, Artificial sequence
  Artificial sequence
ttcatcttccaaggccaatc

SEQ ID NO: 12 - DNA, 20 bp, Artificial sequence
  Artificial sequence
gggctgaacctggtagacag

SEQ ID NO: 13 - DNA, 22 bp, Artificial sequence
  Artificial sequence
ttgagtttggaaacatctggag

SEQ ID NO: 14 - DNA, 21 bp, Artificial sequence
  Artificial sequence
gcccaaagggaactgatagtc